European Patent Specification EP 3 601 618 B1, published September 4, 2024. Title: COMPOSITIONS, METHODS AND KITS TO DETECT ADENOVIRUS, METAPNEUMOVIRUS, AND/OR RHINOVIRUS NUCLEIC ACIDS. Applicant: GEN-PROBE INCORPORATED MAJLESSI, Mehrdad HILLIUS, Amber DOUGLASS, Pamela SHAH, Ankur KOLK, Daniel. Application TBA. The sequence listing filed with the application follows.

SEQUENCE LISTING (178 sequences)

SEQ ID NO: 1 - DNA, 23 bp, Artificial Sequence
  Synthetic Oligonucleotide
caggacgcctcggrgtayctsag

SEQ ID NO: 2 - DNA, 17 bp, Artificial Sequence
  Synthetic Oligonucleotide
ggagccacvgtgggrtt

SEQ ID NO: 3 - DNA, 17 bp, Artificial Sequence
  Synthetic Oligonucleotide
aaycccacbgtggctcc

SEQ ID NO: 4 - DNA, 24 bp, Artificial Sequence
  Synthetic Oligonucleotide
ccgggtctggtgcagtttgcccgc

SEQ ID NO: 5 - DNA, 17 bp, Artificial Sequence
  Synthetic Oligonucleotide
cacatcgccggacagga

SEQ ID NO: 6 - DNA, 21 bp, Artificial Sequence
  Synthetic Oligonucleotide
catactgaagtaggtgtctgt

SEQ ID NO: 7 - DNA, 21 bp, Artificial Sequence
  Synthetic Oligonucleotide
acagacacctacttcagtatg

SEQ ID NO: 8 - DNA, 17 bp, Artificial Sequence
  Synthetic Oligonucleotide
cggtggtcacatcgtgg

SEQ ID NO: 9 - DNA, 17 bp, Artificial Sequence
  Synthetic Oligonucleotide
ccacgatgtgaccaccg

SEQ ID NO: 10 - DNA, 23 bp, Artificial Sequence
  Synthetic Oligonucleotide
agtacctcagtccgggtctggtg

SEQ ID NO: 11 - DNA, 18 bp, Artificial Sequence
  Synthetic Oligonucleotide
atggctaccccttcgatg

SEQ ID NO: 12 - DNA, 17 bp, Artificial Sequence
  Synthetic Oligonucleotide
accccmtcgatgatgcc

SEQ ID NO: 13 - DNA, 17 bp, Artificial Sequence
  Synthetic Oligonucleotide
gcgggcgaattgcacca

SEQ ID NO: 14 - DNA, 17 bp, Artificial Sequence
  Synthetic Oligonucleotide
tggtgcaattcgcccgc

SEQ ID NO: 15 - DNA, 17 bp, Artificial Sequence
  Synthetic Oligonucleotide
gcgggcaaaytgcacca

SEQ ID NO: 16 - DNA, 17 bp, Artificial Sequence
  Synthetic Oligonucleotide
tggtgcartttgcccgc

SEQ ID NO: 17 - DNA, 24 bp, Artificial Sequence
  Synthetic Oligonucleotide
gactcaggtactccgaagcatcct

SEQ ID NO: 18 - DNA, 24 bp, Artificial Sequence
  Synthetic Oligonucleotide
aggatgcttcggagtacctgagtc

SEQ ID NO: 19 - DNA, 22 bp, Artificial Sequence
  Synthetic Oligonucleotide
ctcaggtactccgaggcgtcct

SEQ ID NO: 20 - DNA, 22 bp, Artificial Sequence
  Synthetic Oligonucleotide
aggacgcctcggagtacctgag

SEQ ID NO: 21 - DNA, 22 bp, Artificial Sequence
  Synthetic Oligonucleotide
ctcaggtactccgaagcatcct

SEQ ID NO: 22 - DNA, 22 bp, Artificial Sequence
  Synthetic Oligonucleotide
aggatgcttcggagtacctgag

SEQ ID NO: 23 - DNA, 20 bp, Artificial Sequence
  Synthetic Oligonucleotide
caggtactccgaggcgtcct

SEQ ID NO: 24 - DNA, 20 bp, Artificial Sequence
  Synthetic Oligonucleotide
aggacgcctcggagtacctg

SEQ ID NO: 25 - DNA, 17 bp, Artificial Sequence
  Synthetic Oligonucleotide
accccatcgatgatgcc

SEQ ID NO: 26 - DNA, 17 bp, Artificial Sequence
  Synthetic Oligonucleotide
accccctcgatgatgcc

SEQ ID NO: 27 - DNA, 17 bp, Artificial Sequence
  Synthetic Oligonucleotide
gcgggcaaactgcacca

SEQ ID NO: 28 - DNA, 17 bp, Artificial Sequence
  Synthetic Oligonucleotide
gcgggcaaattgcacca

SEQ ID NO: 29 - DNA, 22 bp, Artificial Sequence
  Synthetic Oligonucleotide
ctcaggtattccgaggcatcct

SEQ ID NO: 30 - DNA, 22 bp, Artificial Sequence
  Synthetic Oligonucleotide
aggatgcctcggaatacctgag

SEQ ID NO: 31 - DNA, 17 bp, Artificial Sequence
  Synthetic Oligonucleotide
accccatcgatgctgcc

SEQ ID NO: 32 - DNA, 17 bp, Artificial Sequence
  Synthetic Oligonucleotide
accccatcgatgatgcc

SEQ ID NO: 33 - DNA, 18 bp, Artificial Sequence
  Synthetic Oligonucleotide
tgggcgtacatgcacatc

SEQ ID NO: 34 - DNA, 19 bp, Artificial Sequence
  Synthetic Oligonucleotide
gtggtcttacatgcacatc

SEQ ID NO: 35 - DNA, 19 bp, Artificial Sequence
  Synthetic Oligonucleotide
gtgggcatacatgcacatc

SEQ ID NO: 36 - DNA, 22 bp, Artificial Sequence
  Synthetic Oligonucleotide
aggatgcttcggagtacctgag

SEQ ID NO: 37 - DNA, 20 bp, Artificial Sequence
  Synthetic Oligonucleotide
aggacgcctcggagtacctg

SEQ ID NO: 38 - DNA, 20 bp, Artificial Sequence
  Synthetic Oligonucleotide
artggkcdtacatgcacatc

SEQ ID NO: 39 - DNA, 20 bp, Artificial Sequence
  Synthetic Oligonucleotide
caggacgcctcggagtacct

SEQ ID NO: 40 - DNA, 22 bp, Artificial Sequence
  Synthetic Oligonucleotide
aggatgcttcggagtacctgag

SEQ ID NO: 41 - DNA, 17 bp, Artificial Sequence
  Synthetic Oligonucleotide
cacgatgtgaccacaga

SEQ ID NO: 42 - DNA, 17 bp, Artificial Sequence
  Synthetic Oligonucleotide
caygatgtgaccacaga

SEQ ID NO: 43 - DNA, 17 bp, Artificial Sequence
  Synthetic Oligonucleotide
cacgaygtgaccacaga

SEQ ID NO: 44 - DNA, 17 bp, Artificial Sequence
  Synthetic Oligonucleotide
cacgatgtgaccacsga

SEQ ID NO: 45 - DNA, 17 bp, Artificial Sequence
  Synthetic Oligonucleotide
cacgatgtgaccacvga

SEQ ID NO: 46 - DNA, 17 bp, Artificial Sequence
  Synthetic Oligonucleotide
caygaygtgaccacvga

SEQ ID NO: 47 - DNA, 2832 bp, Human adenovirus type 9
  ref <308>: AB330090.1
  ref <309>: 2008-06-14
  ref <313>: (1)..(2832)
atggccaccccctcgatgatgccgcagtgggcgtacatgcacatcgccgggcaggacgcctcggagtacctgagcccgggtctggtgcagtttgcccgcgccaccgacacgtacttcagcctgggcaacaagtttaggaaccccacggtggccccgacccacgatgtgaccacggaccggtcccagcgtctgacgctgcgcttcgtgcccgtggatcgcgaggacaccacgtactcgtacaaggcgcgcttcactctggccgtgggcgacaaccgggtgctagacatggccagcacttactttgacatccgcggcgtcctggaccgcggtcccagcttcaaaccctactcgggcacagcttacaacagtctggcccccaagggtgcccccaactccagccagtggcttgcaaaagacaccaatgctggcgatcaagcattaaaaacccacacacatggcgtagctgctatggggggaacagatatcacagcaaagggtttgcaaattggtgttgacacgactgaaaacaagaatgagcctatttatgcaaatgaaatataccagccagaacctcaggtaggagaggaaaacttgcaagatgttgaaaacttttatggaggcagagctcttaaaaaagaaaccaaaatgaaaccttgctatggctcgtttgccagacccacaaatgaaaaaggcggtcaagccaaatttttaactgacggcgatggtcagctaactaaaaatcatgatatcacaatgaatttctttgacactcctggaggaacagttggtcaggatactgaacttgaagcagacattgttatgtatgctgagaatgtgcatctggaaactccagacacgcatgtggtgtacaaaccaggaacttctgatgagagttcagaagcaaatttggttcagcagtccatgccaaacaggcccaactacatcggcttcagggacaactttgtgggtctcatgtactataacagcactggcaacatgggtgtgctggctggtcaagcatctcagttgaatgctgtggtcgacttgcaagacagaaacacagagctgtcttaccagctcttgctagattctctgggtgacagaaccagatactttagcatgtggaactctgcagtggacagttatgatcctgatgtcaggattattgaaaatcacggtgtggaagatgaacttccaaactattgcttcccattggatggagctggcactaatgctacctaccaaggtgtaaaagttaaaaatggccaagatggagatgtaaacgcagattgggaaaaagatccaaatcttgcttcacgaaaccaaatatgcaagggtaacatcttcgccatggagatcaacctccaggccaacctgtggaagagttttctgtactcgaatgtggccctgtacctgcccgactcatacaagtacacgccggccaacgtcacgctgcccgccaataccaacacctacgagtacatgaacggccgcgtggtagccccctcgctggtggacgcctacatcaacatcggcgcccggtggtcgctggaccccatggacaacgtcaacccattcaaccaccaccgcaacgcgggcctgcgttaccgctccatgcttctgggcaacggccgctacgtgcccttccacatccaagtgccccaaaagttctttgccatcaagaacctgctcctgctccccggctcctacacctacgagtggaacttccgcaaggatgtcaacatgatcctgcagagttccctcggaaacgacctgcgcgtcgacggcgcctccgtccgcttcgacagcgtcaacctctacgccacattcttccccatggcgcacaacaccgcctccaccctggaagccatgctgcgcaacgacaccaacgaccagtccttcaacgactacctctcggccgccaacatgctctaccccatcccggccaaggccaccaacgtgcccatctccatcccctcgcgcaactgggccgccttccgcggctggagtttcacccggctcaagaccaaagaaactccctccctcggctcgggtttcgatccctactttgtatactcgggttccatcccctacctcgacgggaccttctacctcaaccacaccttcaagaaggtctccatcatgttcgactcctcggtcagctggcccggcaacgaccggctgctcacgccgaacgagttcgagatcaagcgcagtgtcgacggggagggctacaatgtggcccaatgcaacatgaccaaggactggttcctcgtccagatgctctcccactacaacatcggctaccagggcttccacgtgcccgagggctacaaggaccgcatgtactccttcttccgcaacttccagcccatgagcaggcaggtggtcgatgagatcaactacaaggactacaaggccgtcaccctgcccttccagcacaacaactcgggcttcaccggctaccttgcacccaccatgcgtcaggggcagccctaccccgccaacttcccctatcctctcatcggccagacagccgtgccctctgtcacccagaaaaagttcctctgcgacagggtcatgtggcgcatccccttctccagcaacttcatgtccatgggcgccctcaccgacctgggtcagaacatgctctatgccaactcggcccacgcgctcgacatgaccttcgaggtggaccccatggatgagcccaccctcctctatcttctcttcgaagttttcgacgtggtcagagtgcaccagccgcaccgcggcgtcatcgaggccgtctacctgcgcacgcccttctccgccggcaacgccaccacctaa

SEQ ID NO: 48 - DNA, 17 bp, Artificial Sequence
  Synthetic Oligonucleotide
agcctgcgtggcggcca

SEQ ID NO: 49 - DNA, 20 bp, Artificial Sequence
  Synthetic Oligonucleotide
agccugcgtggtgcccugcc

SEQ ID NO: 50 - DNA, 22 bp, Artificial Sequence
  Synthetic Oligonucleotide
cactagtutggtcgatgaggct

SEQ ID NO: 51 - DNA, 27 bp, Artificial Sequence
  Synthetic Oligonucleotide
ccatctgtagattaggguaatgaggct

SEQ ID NO: 52 - DNA, 26 bp, Artificial Sequence
  Synthetic Oligonucleotide
cccaactttgcaagtgttgttctcgg

SEQ ID NO: 53 - DNA, 27 bp, Artificial Sequence
  Synthetic Oligonucleotide
ccccaattttgctagtgttgttcttgg

SEQ ID NO: 54 - DNA, 17 bp, Artificial Sequence
  Synthetic Oligonucleotide
ccugcgtggctgcctgc

SEQ ID NO: 55 - DNA, 28 bp, Artificial Sequence
  Synthetic Oligonucleotide
cgtcgaccgaagtcctgcaaaaggtcac

SEQ ID NO: 56 - DNA, 28 bp, Artificial Sequence
  Synthetic Oligonucleotide
ctgctgctgaaaatagttctgtgtttgg

SEQ ID NO: 57 - DNA, 23 bp, Artificial Sequence
  Synthetic Oligonucleotide
gaaacacggacacccaaagtagt

SEQ ID NO: 58 - DNA, 21 bp, Artificial Sequence
  Synthetic Oligonucleotide
ggcctctgctaaagcaacacc

SEQ ID NO: 59 - DNA, 21 bp, Artificial Sequence
  Synthetic Oligonucleotide
gtagatcggggcaatggggct

SEQ ID NO: 60 - DNA, 21 bp, Artificial Sequence
  Synthetic Oligonucleotide
gtagatcggggtaatggggct

SEQ ID NO: 61 - DNA, 18 bp, Artificial Sequence
  Synthetic Oligonucleotide
gtggcgcgggcgaactgc

SEQ ID NO: 62 - DNA, 18 bp, Artificial Sequence
  Synthetic Oligonucleotide
gttgcacgggcgaactgc

SEQ ID NO: 63 - DNA, 23 bp, Artificial Sequence
  Synthetic Oligonucleotide
tacatgcacatcgccgggcagga

SEQ ID NO: 64 - DNA, 23 bp, Artificial Sequence
  Synthetic Oligonucleotide
tacatgcacatctcgggccagga

SEQ ID NO: 65 - DNA, 19 bp, Artificial Sequence
  Synthetic Oligonucleotide
tagacctggcagatgaggc

SEQ ID NO: 66 - DNA, 19 bp, Artificial Sequence
  Synthetic Oligonucleotide
tgccgcagaacgttgcgaa

SEQ ID NO: 67 - DNA, 33 bp, Artificial Sequence
  Synthetic Oligonucleotide
tgcctcaggcttaggcataataggtatgtatcg

SEQ ID NO: 68 - DNA, 27 bp, Artificial Sequence
  Synthetic Oligonucleotide
tgctgcagaaaatagctctgtgtttgg

SEQ ID NO: 69 - DNA, 33 bp, Artificial Sequence
  Synthetic Oligonucleotide
tgcttcaggtctaggtataatcggaatgtacag

SEQ ID NO: 70 - DNA, 33 bp, Artificial Sequence
  Synthetic Oligonucleotide
tgcttcaggtttaggcataatcggaatgtacag

SEQ ID NO: 71 - DNA, 20 bp, Artificial Sequence
  Synthetic Oligonucleotide
tggccactccgtcgatgatg

SEQ ID NO: 72 - DNA, 20 bp, Artificial Sequence
  Synthetic Oligonucleotide
tggctaccccatcgatgatg

SEQ ID NO: 73 - DNA, 20 bp, Artificial Sequence
  Synthetic Oligonucleotide
tggctaccccatcgatgctg

SEQ ID NO: 74 - DNA, 20 bp, Artificial Sequence
  Synthetic Oligonucleotide
tggctaccccutcgatgatg

SEQ ID NO: 75 - DNA, 20 bp, Artificial Sequence
  Synthetic Oligonucleotide
ctagtutggtcgatgaggct

SEQ ID NO: 76 - DNA, 425 bp, Human rhinovirus
  ref <308>: HM581865.1
  ref <309>: 2010-09-09
  ref <313>: (1)..(425)
ggtgtgtgaatagactctaacagggttgaagctgtagcactcgttatccgcacaactactacgcgaatgttagtaacaccctctaggtatagtgggatttcgctccgcagaaaccccatctgtagattagggtaatgaggctacacagaccccactggcgacagtggtgtagcctgcgtggtgccctacctggggtttctcaccccaggattccactttactgacagggtgtgaaggcgctagtgtgctagttgtgagtcctccggtccctgaatgtggctaatcctaaccccgtggccatttcatgtaatccaacatgcaggtggtcgtaacgagcaatcacgggatggaaccaactactttgggtaaccgtgtttcctgttttactttaatgtgtgtcttatggttacaattatagagtaacc

SEQ ID NO: 77 - DNA, 29 bp, Artificial Sequence
  Synthetic Oligonucleotide
ccatctgtagrtyrgggyaatgrggctac

SEQ ID NO: 78 - DNA, 23 bp, Artificial Sequence
  Synthetic Oligonucleotide
gtagattaggguaatgaggctac

SEQ ID NO: 79 - DNA, 21 bp, Artificial Sequence
  Synthetic Oligonucleotide
gtagattaggguaatgaggct

SEQ ID NO: 80 - DNA, 21 bp, Artificial Sequence
  Synthetic Oligonucleotide
gtagatcrggguaatggggct

SEQ ID NO: 81 - DNA, 21 bp, Artificial Sequence
  Synthetic Oligonucleotide
gtagatcrgggyaatggggct

SEQ ID NO: 82 - DNA, 21 bp, Artificial Sequence
  Synthetic Oligonucleotide
gtagatcrggguaatgrggct

SEQ ID NO: 83 - DNA, 23 bp, Artificial Sequence
  Synthetic Oligonucleotide
gtagatcggggtaatggggctac

SEQ ID NO: 84 - DNA, 23 bp, Artificial Sequence
  Synthetic Oligonucleotide
gtagatcggggcaatggggctac

SEQ ID NO: 85 - DNA, 19 bp, Artificial Sequence
  Synthetic Oligonucleotide
gtagatcrgggyaatgrgg

SEQ ID NO: 86 - DNA, 23 bp, Artificial Sequence
  Synthetic Oligonucleotide
gtagatcrgggyaatgrggctac

SEQ ID NO: 87 - DNA, 20 bp, Artificial Sequence
  Synthetic Oligonucleotide
agcctgcgtggyksccwrcc

SEQ ID NO: 88 - DNA, 20 bp, Artificial Sequence
  Synthetic Oligonucleotide
agccygcgtggtgcccygcc

SEQ ID NO: 89 - DNA, 17 bp, Artificial Sequence
  Synthetic Oligonucleotide
cugcgtggtgcccygcc

SEQ ID NO: 90 - DNA, 17 bp, Artificial Sequence
  Synthetic Oligonucleotide
cygcgtggtgcccugcc

SEQ ID NO: 91 - DNA, 14 bp, Artificial Sequence
  Synthetic Oligonucleotide
agccygcgtggtgc

SEQ ID NO: 92 - DNA, 17 bp, Artificial Sequence
  Synthetic Oligonucleotide
agcctgcgtggcggcca

SEQ ID NO: 93 - DNA, 16 bp, Artificial Sequence
  Synthetic Oligonucleotide
agccygcgtggtgccc

SEQ ID NO: 94 - DNA, 17 bp, Artificial Sequence
  Synthetic Oligonucleotide
ccugcgtggctgcctgc

SEQ ID NO: 95 - DNA, 27 bp, Artificial Sequence
  Synthetic Oligonucleotide
grttagccrcattcaggggccggagga

SEQ ID NO: 96 - DNA, 35 bp, Artificial Sequence
  Synthetic Oligonucleotide
gaaacacggacacccaaagtagtyggtyccrtccc

SEQ ID NO: 97 - DNA, 19 bp, Artificial Sequence
  Synthetic Oligonucleotide
aagtagttggtcccatccc

SEQ ID NO: 98 - DNA, 19 bp, Artificial Sequence
  Synthetic Oligonucleotide
aagtagttggttccatccc

SEQ ID NO: 99 - DNA, 19 bp, Artificial Sequence
  Synthetic Oligonucleotide
aagtagtcggtcccatccc

SEQ ID NO: 100 - DNA, 19 bp, Artificial Sequence
  Synthetic Oligonucleotide
aagtagttggtcccgtccc

SEQ ID NO: 101 - DNA, 549 bp, Human rhinovirus
  ref <308>: EU096024.1
  ref <309>: 2008-02-15
  ref <313>: (1)..(549)
ttcctaatgtacccaccctaaaacttcctacccaagtaacgttagaagtttcatcaacaagtacaataggaagcatcacatccagtggtgttttgtacaagcacttctgtttccccggagcgaggtataggctgtacccactgccgaaagcctttaaccgttatccgccaaccaactacgtaaaagctagtatcatcatgttttaaaataggcgttcgatcaggtggatcccccctccactagtttggtcgatgaggctaggaactccccacgggtgaccgtgtcctagcctgcgtggcggccaacccagcttctgctgggacgcctttttatggacatggtgtgaagactcgcatgtgcttggttgtgactcctccggcccctgaatgcggctaaccttaaccccggagccctgtgttgcaatccagtaacattagggtcgtaatgagcaatttcgggacgggaccgactactttgggtgtccgtgtttctcatttttcttattattgtcttatggtcacagcatatatataacgtatatactgtgat

SEQ ID NO: 102 - DNA, 22 bp, Artificial Sequence
  Synthetic Oligonucleotide
cactagtttggycgatgaggct

SEQ ID NO: 103 - DNA, 19 bp, Artificial Sequence
  Synthetic Oligonucleotide
ctagtytggtcgatgaggc

SEQ ID NO: 104 - DNA, 18 bp, Artificial Sequence
  Synthetic Oligonucleotide
ctagtytggtcgatgagg

SEQ ID NO: 105 - DNA, 16 bp, Artificial Sequence
  Synthetic Oligonucleotide
gtytggtcgatgaggc

SEQ ID NO: 106 - DNA, 19 bp, Artificial Sequence
  Synthetic Oligonucleotide
tagtytggtcgatgaggct

SEQ ID NO: 107 - DNA, 19 bp, Artificial Sequence
  Synthetic Oligonucleotide
tagtutggtcgatgaggct

SEQ ID NO: 108 - DNA, 18 bp, Artificial Sequence
  Synthetic Oligonucleotide
rcattcaggggccggagg

SEQ ID NO: 109 - DNA, 20 bp, Artificial Sequence
  Synthetic Oligonucleotide
agcctgcgtggcggccarcc

SEQ ID NO: 110 - DNA, 17 bp, Artificial Sequence
  Synthetic Oligonucleotide
ccugcgtggctgcctrc

SEQ ID NO: 111 - DNA, 17 bp, Artificial Sequence
  Synthetic Oligonucleotide
ctgcgtggtgccctacc

SEQ ID NO: 112 - DNA, 17 bp, Artificial Sequence
  Synthetic Oligonucleotide
ccygcgtggctgcctac

SEQ ID NO: 113 - DNA, 14 bp, Artificial Sequence
  Synthetic Oligonucleotide
agccygcgtggctg

SEQ ID NO: 114 - DNA, 16 bp, Artificial Sequence
  Synthetic Oligonucleotide
agccygcgtggctgcc

SEQ ID NO: 115 - DNA, 27 bp, Artificial Sequence
  Synthetic Oligonucleotide
grttagccrcattcrggrgccggagga

SEQ ID NO: 116 - DNA, 18 bp, Artificial Sequence
  Synthetic Oligonucleotide
gcattcaggggccggagg

SEQ ID NO: 117 - DNA, 26 bp, Artificial Sequence
  Synthetic Oligonucleotide
gaaacacggacacccaaagtagtygg

SEQ ID NO: 118 - DNA, 29 bp, Artificial Sequence
  Synthetic Oligonucleotide
gaaacacggacacccaaagtagtyggtcc

SEQ ID NO: 119 - DNA, 19 bp, Artificial Sequence
  Synthetic Oligonucleotide
aagtagtcggtcccgtccc

SEQ ID NO: 120 - DNA, 576 bp, Human rhinovirus
  ref <308>: EU095989.1
  ref <309>: 2008-02-15
  ref <313>: (1)..(576)
tggatttcccacaggagtggtactctgttattacggtaactttgtacgccagttttatctcccttcccccatgtaacttagaagtttttcacaaagaccaatagccggtaatcagccagattactgaaggtcaagcacttctgtttccccggtcaatgttgatatgctccaacagggcaaaaacaactgcgatcgttatccgcaaagcgcctacgcaaagcttagtagcatctttgaaatcgtttggctggtcgatccgccatttcccctggtagacctggcagatgaggctagaaataccccactggcgacagtgttctagcctgcgtggctgcctgcacaccctatgggtgtgaagccaaacaatggacaaggtgtgaagagccccgtgtgctcgctttgagtcctccggcccctgaatgtggctaaccttaaccctgcagctagagcacgtaacccaacgtgtatctagtcgtaatgagcaattgcgggatgggaccaactactttgggtgtccgtgtttcactttttcctttatatttgcttatggtgacaatatatacaatatatatattg

SEQ ID NO: 121 - DNA, 19 bp, Artificial Sequence
  Synthetic Oligonucleotide
yrgrcytggcagatgrggc

SEQ ID NO: 122 - DNA, 19 bp, Artificial Sequence
  Synthetic Oligonucleotide
taracctggcagatgrggc

SEQ ID NO: 123 - DNA, 19 bp, Artificial Sequence
  Synthetic Oligonucleotide
tagacctggcagatggggc

SEQ ID NO: 124 - DNA, 19 bp, Artificial Sequence
  Synthetic Oligonucleotide
tagacctggcagatgrggc

SEQ ID NO: 125 - DNA, 19 bp, Artificial Sequence
  Synthetic Oligonucleotide
taracctggcagatggggc

SEQ ID NO: 126 - DNA, 19 bp, Artificial Sequence
  Synthetic Oligonucleotide
taracctggtagatgrggc

SEQ ID NO: 127 - DNA, 17 bp, Artificial Sequence
  Synthetic Oligonucleotide
taracctggcagatgrg

SEQ ID NO: 128 - DNA, 18 bp, Artificial Sequence
  Synthetic Oligonucleotide
taracctggcagatgrgg

SEQ ID NO: 129 - DNA, 19 bp, Artificial Sequence
  Synthetic Oligonucleotide
caracctggcagatgrggc

SEQ ID NO: 130 - DNA, 15 bp, Artificial Sequence
  Synthetic Oligonucleotide
cctgccagatgrggc

SEQ ID NO: 131 - DNA, 19 bp, Artificial Sequence
  Synthetic Oligonucleotide
wgcctgcgyggckgccwrc

SEQ ID NO: 132 - DNA, 17 bp, Artificial Sequence
  Synthetic Oligonucleotide
ccygcgcggctgcctrc

SEQ ID NO: 133 - DNA, 17 bp, Artificial Sequence
  Synthetic Oligonucleotide
ccygcgtggctgcctrc

SEQ ID NO: 134 - DNA, 17 bp, Artificial Sequence
  Synthetic Oligonucleotide
ccygcgtggctgcctgc

SEQ ID NO: 135 - DNA, 19 bp, Artificial Sequence
  Synthetic Oligonucleotide
wgccygcgtggctgcctgc

SEQ ID NO: 136 - DNA, 19 bp, Artificial Sequence
  Synthetic Oligonucleotide
agccygcgtggctgcctgc

SEQ ID NO: 137 - DNA, 27 bp, Artificial Sequence
  Synthetic Oligonucleotide
grttagccgcattcrggrgccggagga

SEQ ID NO: 138 - DNA, 46 bp, Artificial Sequence
  Synthetic Oligonucleotide
tacatgcacatckcsggvcaggaygcytcggagtacctgagccccg

SEQ ID NO: 139 - DNA, 22 bp, Artificial Sequence
  Synthetic Oligonucleotide
acgcctcggagtacctgagccc

SEQ ID NO: 140 - DNA, 24 bp, Artificial Sequence
  Synthetic Oligonucleotide
cggggctcaggtactccgaggcgt

SEQ ID NO: 141 - DNA, 22 bp, Artificial Sequence
  Synthetic Oligonucleotide
gtkgcrcgggcraaytgcacca

SEQ ID NO: 142 - DNA, 18 bp, Artificial Sequence
  Synthetic Oligonucleotide
gtkgcrcgggcgaactgc

SEQ ID NO: 143 - DNA, 17 bp, Artificial Sequence
  Synthetic Oligonucleotide
gtggcgcgggcaaactg

SEQ ID NO: 144 - DNA, 18 bp, Artificial Sequence
  Synthetic Oligonucleotide
gtkgcrcgggcraactgc

SEQ ID NO: 145 - DNA, 18 bp, Artificial Sequence
  Synthetic Oligonucleotide
gtggcrcgggcraactgc

SEQ ID NO: 146 - DNA, 18 bp, Artificial Sequence
  Synthetic Oligonucleotide
gtkgcgcgggcraactgc

SEQ ID NO: 147 - DNA, 18 bp, Artificial Sequence
  Synthetic Oligonucleotide
gtggcgcgggcraactgc

SEQ ID NO: 148 - DNA, 18 bp, Artificial Sequence
  Synthetic Oligonucleotide
gtggcrcgggcgaactgc

SEQ ID NO: 149 - DNA, 18 bp, Artificial Sequence
  Synthetic Oligonucleotide
gtkgcgcgggcgaactgc

SEQ ID NO: 150 - DNA, 13293 bp, Human Metapneumovirus
  ref <308>: AY525843.1
  ref <309>: 2008-02-15
  ref <313>: (1)..(13293)
acgcgaaaaaaacgcgtataaattaaattccaaacaaaacgggacaaataaaaatgtctcttcaagggattcacctaagtgatctatcatataaacatgctatattaaaagagtctcaatacacaataaaaagagatgtaggcaccacaactgcagtgacaccttcatcattacaacaagaaataacacttttgtgtggggaaatactttacactaaacacactgattacaaatatgctgctgagataggaatacaatatatttgcacagctctaggatcagaaagagtacaacagattttgagaaactcaggtagtgaagttcaggtggttctaaccaaaacatactccttagggaaaggcaaaaacagtaaaggggaagagctgcagatgttagatatacatggagtggaaaagagttggatagaagaaatagacaaagaggcaagaaagacaatggtaactttgcttaaggaatcatcaggtaacatcccacaaaaccagagaccttcagcaccagacacaccaataattttattatgtgtaggtgccctaatattcactaaactagcatcaacaatagaagttggattagagactacagttagaagagctaatagagtgctaagtgatgcactcaaaagatacccaaggatagatataccaaagattgctagatctttttatgaactatttgaacaaaaagtgtactacagaagtttattcattgagtacggaaaagctttaggctcatcttcaacaggaagcaaagcagaaagtttgtttgtaaatatatttatgcaagcttatggagctggccaaacactgctaaggtggggtgtcattgccagatcatccaacaacataatgctagggcatgtatctgtgcaatctgaattgaagcaagttacagaggtttatgacttggtgagagaaatgggtcctgaatctgggcttttacatctaagacaaagtccaaaggcagggctgttatcattggccaattgccccaattttgctagtgttgttcttggcaatgcttcaggtctaggcataatcggaatgtacagagggagagtaccaaacacagagctattttctgcagcagaaagttatgccagaagcttaaaagaaagcaataaaatcaacttctcttcgttagggcttacagatgaagaaaaagaagctgcagaacacttcttaaacatgagtggtgacaatcaagatgattatgagtaattaaaaaactgggacaagtcaaaatgtcattccctgaaggaaaggatattctgttcatgggtaatgaagcagcaaaaatagccgaagctttccagaaatcactgaaaaaatcaggtcacaagagaactcaatctattgtaggggaaaaagttaacactatatcagaaactctagaactacctaccatcagcaaacctgcacgatcatctacactgctggaaccaaaattggcatgggcagacaacagcggaatcaccaaaatcacagaaaaaccagcaaccaaaacaacagatcctgttgaagaagaggaattcaatgaaaagaaagtgttaccttccagtgatgggaagactcctgcagagaaaaaatcaaagttttcaaccagtgtaaaaaagaaagtttcctttacatcaaatgaaccagggaaatacaccaaactagagaaagatgccctagatttgctctcagacaatgaggaagaagacgcagaatcctcaatcctaacttttgaggagaaagatacatcatcactaagcattgaagctagactagaatctatagaagagaagttgagcatgatattaggactgcttcgtacacttaacattgcaacagcaggaccaacagctgcacgagatggaattagggatgcaatgattggtataagagaagagctaatagcagagataattaaggaagccaagggaaaagcagctgaaatgatggaagaagagatgaatcaaagatcaaaaataggaaatggcagtgtaaaactaaccgagaaggcaaaagagctcaacaaaattgttgaagacgagagcacaagcggtgaatcagaagaagaagaagaaccaaaagaaactcaggataacaatcaaggagaagatatttatcagttaatcatgtagtttaataaaaataaacaatgggacaagtcaagatggagtcctatctagtagacacttatcaaggcattccatatacagctgctgttcaagttgacctggtagaaaaagatttactgccagcaagtttgacaatatggtttcctttatttcaggccaacacaccaccagcagttctgcttgatcagctaaaaaccttgacaataacaactctgtatgctgcatcacagaatggtccaatactcaaggtaaatgcatctgcccaaggtgctgccatgtctgtacttcccaaaaaattcgaggtaaatgcaactgtagcacttgatgaatacagtaaacttgattttgacaagctgacggtctgcgatgttaaaacagtttatttgacaactatgaaaccgtacgggatggtgtcaaaatttgtgagttcagccaaatcagttggcaaaaagacacatgatctaattgcactatgtgacttcatggacctagagaaaaatatacctgtgacaataccagcattcataaagtcagtttcaatcaaagagagtgaatcagccactgttgaagctgcaataagcagcgaagccgaccaagccttgacacaagccaagattgcgccctatgcaggactaattatgatcatgaccatgaacaatccaaaaggtatattcaagaaactaggggctggaacacaagtgatagtagagctgggggcatatgttcaggctgagagcatcagtaggatctgcaagagctggagtcaccaaggaacaagatacgtactaaaatccagataaaaataactgtcttaatcaataattgcttatataactctagagattaataagcttattattatagttatataaaaataaattagaattagaagggcatcaatagaaagcgggacaaataaaaatgtcttggaaagtgatgatcatcatttcgttactcataacaccccagcacgggctaaaggagagttatttggaagaatcatgtagtactataactgagggatacctcagtgttttaagaacaggctggtacactaatgtcttcacattagaagttggtgatgttgaaaatcttacatgtactgatggacctagcttaatcaaaacagaacttgatctaacaaaaagtgctttaagggaactcaaaacagtctctgctgatcagttggcgagagaggagcaaattgaaaatcccagacaatcaagatttgtcttaggtgcgatagctctcggagttgctacagcagcagcagtcacagcaggcattgcaatagccaaaaccataaggcttgagagtgaggtgaatgcaattaaaggtgctctcaaacaaactaatgaagcagtatccacattagggaatggtgtgcgggtcctagccactgcagtgagagagctaaaagaatttgtgagcaaaaacctgactagtgcaatcaacaggaacaaatgtgacattgctgatctgaagatggctgtcagcttcagtcaattcaacagaagatttctaaatgttgtgcggcagttttcagacaatgcagggataacaccagcaatatcattggacctgatgactgatgctgagttggccagagctgtatcatacatgccaacatctgcagggcagataaaactgatgttggagaaccgcgcaatggtaaggagaaaaggatttggaatcctgataggggtctacggaagctctgtgatttacatggttcaattgccgatctttggtgtcatagatacaccttgttggatcatcaaggcagctccctcttgctcagaaaaaaacgggaattatgcttgcctcctaagagaggatcaagggtggtattgtaaaaatgcaggatctactgtttactacccaaatgaaaaagactgcgaaacaagaggtgatcatgttttttgtgacacagcagcagggatcaatgttgctgagcaatcaagagaatgcaacatcaacatatctactaccaactacccatgcaaagtcagcacaggaagacaccctataagcatggttgcactatcacctctcggtgctttggtggcttgctataaaggggtaagctgctcgattggcagcaattgggttggaatcatcaaacaattacccaaaggctgctcatacataaccaaccaggatgcagacactgtaacaattgacaataccgtgtatcaactaagcaaagttgaaggtgaacagcatgtaataaaagggagaccagtttcaagcagttttgatccaatcaagtttcctgaggatcagttcaatgttgcgcttgatcaagtcttcgaaagcattgagaacagtcaggcactagtggaccagtcaaacaaaattctaaacagtgcagaaaaaggaaacactggtttcattatcgtagtaattttggttgctgttcttggtctaaccatgatttcagtgagcatcatcatcataatcaagaaaacaaggaagcccacaggagcacctccagagctgaatggtgtcaccaacggcggtttcataccacatagttagttaattaaaaaatgggacaaatcatcatgtctcgtaaggctccatgcaaatatgaagtgcggggcaaatgcaacagagggagtgattgcaaattcaatcacaattactggagttggcctgatagatatttattgttaagatcaaattatctcttaaatcagcttttaagaaacacagataaggctgatggtttgtcaataatatcaggagcaggtagagaagatagaactcaagactttgttcttggttctactaatgtggttcaagggtacattgatgacaaccaaggaataaccaaggctgcagcttgctatagtctacacaacataatcaagcaactacaagaaacagaagtaagacaggctagagacaacaagctttctgatagcaaacatgtggcgctccacaacttgatattatcctatatggagatgagcaaaactcctgcatctctaatcaacaacctaaagaaactaccaagggaaaaactgaagaaattagcaagattaataattgatttatcagcaggaactgacaatgactcttcatatgccttgcaagacagtgaaagcactaatcaagtgcagtaaacatggtcccaaattcattaccatagaggcagatgatatgatatggactcacaaagaattaaaagaaacactgtctgatgggatagtaaaatcacacaccaatatttatagttgttacttagaaaatatagaaataatatatgttaaaacttacttaagttagtaaaaaataaaaatagaatgggataaatgacaatgaaaacattagatgtcataaaaagtgatggatcctcagaaacgtgtaatcaactcaaaaaaataataaaaaaacactcaggtaaagtgcttattgcactaaaactgatattggccttactgacatttttcacagcaacaatcactgtcaactatataaaagtagaaaacaatttgcaggcatgtcaaccaaaaaatgaatcagacaaaaaggtcacaaagccaaataccacatcaacaacaatcagacccacacccgatccaactgtagtacatcatttgaaaaggctgattcagagacacaccaactctgtcacaaaagacagcgatacttgttggagaatacacaagaatcaacgtacaaatataaaaatatacaagttcttatgctctgggttcacaaattcaaaaggtacagattgtgaggaaccaacagccctatgcgacaaaaagttaaaaaccatagtagaaaaacatagaaaagcagaatgtcactgtctacatacaaccgagtgggggtgccttcatccctaaaataacacggctttcaacattaaaatcagaacaacctccacccaggtctatcaatacagtggtttagccatttaaaaaccgaatattatctaggctgcacgacactttgcaataatatgcaatagtcaatagttaaaccactgctgcaaactcatccataatataatcactgagtaatacaaaacaagaaaatgggacaagtggctatggaagtaagagtggagaacattcgagcgatagacatgttcaaagcaaagataaaaaaccgtataagaagcagcaggtgctatagaaatgctacactgatccttattggactaacagcgttaagcatggcacttaatattttcctgatcatcgatcatgcaacattaagaaacatgatcaaaacagaaaactgtgctaacatgccgtcggcagaaccaagcaaaaagaccccaatgacctccacagcaggcccaaacaccaaacccaatccacagcaagcaacacagtggaccacagagaactcaacatccccagtagcaaccccagagggccatccatacacagggacaactcaaacatcagacacaacagctccccagcaaaccacagacaaacacacagcaccgctaaaatcaaccaatgaacagatcacccagacaaccacagagaaaaagacaatcagagcaacaacccaaaaaagggaaaaaggaaaagaaaacacaaaccaaaccacaagcacagctgcaacccaaacaaccaacaccaccaaccaaatcagaaatgcaagtgagacaatcacaacatccgacagacccagaactgacaccacaacccaaagcagcgaacagacaacccgggcaacagacccaagctccccaccacaccatgcatagagaggtgcaaaactcaaatgagcacaacacacaaacatcccatccaagtagttaacaaaaaaccacaaaataaccttgaaaaccaaaaaaccaaaacataaacccagacccagaaaaacatagacaccatatggaaggttctagcatatgcaccaatgagatggcatctgttcatgtatcaatagcaccaccatcattcaaggaataagaagaggcgaaaatttaagggataaatgacaatggatcccttttgtgaatctactgttaatgtttatctccctgattcatatctcaaaggagtaatatcttttagtgaaaccaatgcaattggatcatgtcttttgaaaagaccctatctaaaaaatgacaacactgccaaagttgctgtagaaaaccctgttgttgaacatgtgaggcttagaaatgcagtcatgaccaaaatgaagatatcagattataaagtggttgaaccagttaatatgcagcatgaaataatgaaaaatatacatagttgtgagcttacattattaaaacaattcttaacgagaagcaaaaacattagctctctaaaattaaatatgatatgtgattggttacagttaaaatccacttcagataacacatcaattctcaattttatagatgtggagttcatacccgtttgggtaagcaattggttcagtaactggtataatctcaataaattaatcttagagtttagaagagaagaagtaataagaactggttcaattttatgtagatcactaggcaagttagtttttattgtatcatcttatggatgtgtagtaaaaagcaacaaaagtaaaagagtgagctttttcacctataaccaactgttaacatggaaagatgtgatgttaagtagattcaatgcaaacttttgtatatgggtaagtaacaacctgaacaaaaatcaagaaggactaggacttagaagcaatctgcaaggtatgttaaccaataaattatatgaaactgttgattacatgctaagcctatgctgcaatgaaggattctctctggtgaaagagtttgaaggatttattatgagtgaaattctaaaaattactgagcatgctcagttcagtactaggtttaggaatactttattgaatgggttaactgaacaattatcagtgttgaaagctaagaacagatctagagttcttggaactatattagaaaacaacaattaccctatgtacgaagtagtacttaaattattaggggacaccttgaaaagcataaagttattaattaacaagaatttagaaaatgctgcagaattatattatatattcagaatttttggacaccctatggtagatgagagggaagcaatggatgctgttaaattaaacaatgagattacaaaaattcttaaattagagagtttaacagaactaagaggagcatttatactaagaattataaaagggtttgtagacaataataaaagatggcctaaaattaagaatttaaaagtgctcagcaaaagatgggctatgtatttcaaagctaaaagttaccctagccaacttgagctaagtgtacaagattttttagaacttgctgcagtacaatttgagcaggaattctctgtacctgaaaaaaccaaccttgagatggtattaaatgataaagcaatatcacctccaaaaaagctaatatggtctgtatatccaaaaaactacctgcctgaaactataaaaaatcaatatttagaagaggctttcaatgcaagtgacagccaaagaacaaggagagtcttagaattttacttaaaagattgtaaatttgatcaaaaagaacttaaacgttatgtaattaaacaagagtatctgaatgacaaagaccacattgtctcgttaactgggaaggaaagagaattaagtgtaggtaggatgtttgcaatgcaaccaggaaaacaaagacagatacagatattagctgagaaacttctagctgataatattgtaccttttttcccagaaactttaacaaagtatggtgacttagatctccaaagaattatggaaataaaatcagaactttcttccattaaaactagaaagaatgatagctacaacaattatattgcaagggcctctatagtaacagacttaagtaagttcaatcaggcctttagatatgaaaccacagctatatgtgcagatgtagctgatgagttacatgggacacaaagcttattctgttggttacatcttattgttcccatgactacaatgatatgtgcatacagacatgcaccaccagaaacaaaaggggaatatgatatagacaaaatacaagagcaaagcggattatacagatatcatatgggagggattgaagggtggtgccagaagttatggacaatggaagcaatatccttgttagatgtagtatctgtgaagactcgctgtcagatgacctctctattaaacggagacaatcagtcaatagatgttagtaaaccagtaaaattgtctgaaggtatagatgaagtaaaagcagactatagcttagcaattagaatgcttaaagaaataagagatgcttataaaaacattggtcataaactcaaagaaggtgaaacatatatatcaagggatctccaatttataagtaaggtgattcaatctgaaggagtcatgcatcctacccctataaaaaagatattaagagtaggtccttggataaatacaatactagatgatattaaaaccagtgcagaatcaataggaagtctatgtcaagaactagaattcagaggggagagtatactagttagcttgatattaaggaatttctggctgtataacttgtacatgtatgagtcaaaacagcacccattagctgggaagcaactgttcaagcaattgaacaaaacattaacatctgtgcagagattttttgaactgaagaaagaaaatgatgtggttgacctatggatgaatataccaatgcagtttggagggggagatccagtagttttttacagatctttttacagaaggactcccgatttcctaactgaagcaatcagccatgtggatttactgttaaaagtgtcaaacaatatcaaagatgagactaagatacgatttttcaaagccttattatctatagaaaagaatgaacgtgctacattaacaacactaatgagagaccctcaggcagtaggatcagaacgacaagctaaggtaacaagtgatataaatagaacagcagttaccagcatactgagtctatctccgaatcagctcttctgtgatagtgctatacattatagtagaaatgaggaagaagttgggatcattgcagacaacataacacctgtctatcctcatgggctgagagtgctctatgaatcactaccttttcataaggctgaaaaggttgtcaatatgatatcaggcacaaagtctataactaatctattacagagaacatctgctatcaatggtgaagatattgatagagcagtgtctatgatgttagagaacttagggttgttatctagaatattgtcagtaataattaatagtatagaaataccaatcaagtccaatggcagattgatatgctgtcaaatttccaagaccttgagagaaaaatcatggaacaatatggaaatagtaggagtgacatctcctagtattgtgacatgtatggatgttgtgtatgcaactagttctcatttaaaaggaataattattgaaaaattcagtactgacaagaccacaagaggtcagaggggaccaaaaagcccctgggtaggatcaagcactcaagagaaaaaattggttcctgtttataatagacaaattctttcaaaacaacaaaaagagcaactggaagcaatagggaaaatgaggtgggtgtacaaaggaactccagggctaagaagattgctcaacaagatttgcataggaagcttaggtattagctataaatgtgtgaaacctttattaccaagattcatgagtgtaaacttcttacataggttatctgttagtagtagacccatggaattcccagcttctgttccagcttacaggacaacaaattaccattttgacactagtccaatcaaccaagcattaagtgagaggttcgggaacgaagacattaatttagtgttccaaaatgcaatcagctgcggaattagtataatgagtgttgtagaacagttaactggtagaagcccaaaacaattagtcctaatccctcaattagaagagatagatattatgcctcctcctgtatttcaaggaaaattcaattataaactagttgataagataacctccgatcaacacatcttcagtcctgacaaaatagacatattaacactagggaagatgcttatgcctaccataaaaggtcaaaaaactgatcagttcttaaataagagagaaaactattttcatggaaataatttaattgaatctttatctgcagcacttgcatgccactggtgtgggatattaacagaacagtgcatagaaaacaatatctttaggaaagattggggtgatgggttcatctcagatcatgccttcatggatttcaaggtatttctatgtgtatttaaaaccaaacttttatgtagttggggatctcaaggaaagaatgtaaaagatgaagatataatagatgaatccattgacaaattattaagaattgacaacaccttttggagaatgttcagcaaagtcatgtttgaatcaaaagtcaaaaaaagaataatgttatatgatgtgaaattcctatcattagtaggttatataggatttaaaaactggtttatagaacagttaagagtggtagaattgcatgaggtaccttggattgtcaatgctgaaggagagttagttgaaattaaatcaatcaaaatttatctgcagttaatagaacaaagtctatctttgagaataactgtattgaattatacagacatggcacatgctcttacacgattaattaggaaaaaattgatgtgtgataatgcactctttaatccaagttcatcaccaatgtttaatctaactcaggttattgatcccacaacacaactagactattttcctaggataatatttgagaggttaaaaagttatgataccagttcagactacaacaaagggaagttaacaaggaattacatgacattattaccatggcaacacgtaaacaggtacaattttgtctttagttctacaggttgtaaagtcagtttgaagacatgcatcgggaaattgataaaggatttaaatcctaaagttctttactttattggagaaggagcaggtaactggatggcaagaacagcatgtgaatatcctgatataaaatttgtatataggagtttaaaggatgaccttgatcaccattacccattagaatatcaaagggtaataggtgatctaaatagggtgatagatagtggtgaaggattatcaatggaaaccacagatgcaactcaaaaaactcattgggacttgatacacagaataagtaaagatgctttattgataacattgtgtgatgcagaattcaaaaacagagatgatttctttaagatggtaatcctttggagaaaacatgtattatcttgtagaatctgtacagcttatggaacagatctttacttatttgcaaagtatcatgcggtggactgcaatataaaattaccattttttgtaagatctgtagctacttttattatgcaaggaagcaaattatcagggtcagaatgttacatacttttaacattaggtcatcacaataatctaccctgtcatggagaaatacaaaattccaaaatgagaatagcagtgtgtaatgatttctatgcctcaaagaaactggacaacaaatcaattgaagcaaactgcaaatctcttctatcaggattgagaatacctataaacaaaaaggagttaaatagacaaaagaaattgttaacactacaaagtaaccattcttctatagcaacagttggcggcagtaagattatagaatccaaatggttaaagaataaagcaagtacaataattgattggttagagcatattttgaattctccaaaaggtgaattaaactatgatttctttgaagcattagagaacacataccccaatatgatcaagcttatagataatttgggaaatgcagaaataaagaaactaatcaaggtcactgggtatatgcttgtgagtaagaagtaataataatgataatgattaaccataatctcacacaactgagaaaataatcgtctaacagtttagttgatcattagttatttaaaattataaaatagtaactaactgataaaaaatcagaaattgaaattgaatgtatacggtttttttgccgt

SEQ ID NO: 151 - DNA, 28 bp, Artificial Sequence
  Synthetic Oligonucleotide
cssccaattttgctagtgttgttcttgg

SEQ ID NO: 152 - DNA, 28 bp, Artificial Sequence
  Synthetic Oligonucleotide
cggccaattttgctagtgttgttcttgg

SEQ ID NO: 153 - DNA, 24 bp, Artificial Sequence
  Synthetic Oligonucleotide
caattttgctagtgttgttcttgg

SEQ ID NO: 154 - DNA, 25 bp, Artificial Sequence
  Synthetic Oligonucleotide
ccaattttgctagtgttgttcttgg

SEQ ID NO: 155 - DNA, 36 bp, Artificial Sequence
  Synthetic Oligonucleotide
tgcttcaggtytaggyataatcggaatgtwcagagg

SEQ ID NO: 156 - DNA, 36 bp, Artificial Sequence
  Synthetic Oligonucleotide
tgcttcaggtttaggcataatcggaatgttcagagg

SEQ ID NO: 157 - DNA, 29 bp, Artificial Sequence
  Synthetic Oligonucleotide
tgcttcaggtctaggtataatcggaatgt

SEQ ID NO: 158 - DNA, 23 bp, Artificial Sequence
  Synthetic Oligonucleotide
gcagaaaatagctctgtgtttgg

SEQ ID NO: 159 - DNA, 1045 bp, Human Metapneumovirus
  ref <308>: JQ309642.1
  ref <309>: 2012-02-12
  ref <313>: (1)..(1045)
cacaataaagagagatgtgggcacaacaacagcagtaacaccctcatcattgcaacaagaaataacactgttgtgtggagaaattctatatgctaagcatactgattacaaatatgctgcagaaataggaatacaatatattagcacagctctagggtcagagagagtacagcagattctaagaaactcaggcagtgaagtccaagcggttttaaccagaacgtactctttggggaaagttaaaaacaataaaggagaagatttacagatgttagacatacatggagtagaaaaaagctgggtggaagagatagacaaagaagcaagaaaaacaatggcaactttacttaaagaatcatcaggcaatattccacaaaatcagaggccttcagcaccagacacacctataatcttattatgtgtaggtgccttaatatttaccaaactagcatcaactatagaagtgggattagagaccacagtcagaagagctaaccgtgtactaagtgatgcactcaaaagataccctagaatggacataccaaaaattgctagatccttctatgacttatttgaacaaaaagtgtatcacagaagtttgttcattgagtatggcaaagcattaggctcatcctctacaggcagcaaagcagaaagtttattcgtcaacatattcatgcaagcttatggtgctggtcaaacaatgctgaggtggggggttatcgccaggtcatctaacaatataatgttaggacatgtatctgtacaagccgagctgaaacaggtcacagaagtctatgacctagtgcgggaaatgggccctgaatctgggctcctacatttaaggcaaagcccaaaagctggactgttatcccttgcaaattgtcccaactttgcaagtgttgttctcggcaatgcctcaggcttaggcataataggtatgtatcgagggagagtgccaaacacagaactattttcagcagcagaaagctatgccaagagtttgaaagaaagtaataaaatcaacttttcttcattaggactc

SEQ ID NO: 160 - DNA, 21 bp, Artificial Sequence
  Synthetic Oligonucleotide
ctttgcaagtgttgttctcgg

SEQ ID NO: 161 - DNA, 37 bp, Artificial Sequence
  Synthetic Oligonucleotide
tgcctcaggcytaggcataatmggyatgtatcghggg

SEQ ID NO: 162 - DNA, 29 bp, Artificial Sequence
  Synthetic Oligonucleotide
tcaggcttaggcataataggtatgtatcg

SEQ ID NO: 163 - DNA, 33 bp, Artificial Sequence
  Synthetic Oligonucleotide
cctcaggcttaggcataataggtatgtatcgag

SEQ ID NO: 164 - DNA, 31 bp, Artificial Sequence
  Synthetic Oligonucleotide
cctcaggcttaggcataataggtatgtatcg

SEQ ID NO: 165 - DNA, 33 bp, Artificial Sequence
  Synthetic Oligonucleotide
cctcaggcttaggcataataggtatgtatcgcg

SEQ ID NO: 166 - DNA, 33 bp, Artificial Sequence
  Synthetic Oligonucleotide
cctcaggcttaggcataataggtatgtatcgug

SEQ ID NO: 167 - DNA, 37 bp, Artificial Sequence
  Synthetic Oligonucleotide
tgcctcaggcctaggcataatcggcatgtatcguggg

SEQ ID NO: 168 - DNA, 37 bp, Artificial Sequence
  Synthetic Oligonucleotide
tgcctcaggcctaggcataatcggcatgtatcgtggg

SEQ ID NO: 169 - DNA, 32 bp, Artificial Sequence
  Synthetic Oligonucleotide
ctcaggcttaggcataataggtatgtatcgcg

SEQ ID NO: 170 - DNA, 34 bp, Artificial Sequence
  Synthetic Oligonucleotide
tgcctcaggcttaggcataataggtatgtatcgc

SEQ ID NO: 171 - DNA, 35 bp, Artificial Sequence
  Synthetic Oligonucleotide
tgcctcaggcttaggcataataggtatgtatcgcg

SEQ ID NO: 172 - DNA, 36 bp, Artificial Sequence
  Synthetic Oligonucleotide
tgcctcaggcttaggcataataggtatgtatcgcgg

SEQ ID NO: 173 - DNA, 37 bp, Artificial Sequence
  Synthetic Oligonucleotide
tgcctcaggcttaggcataataggtatgtatcguggg

SEQ ID NO: 174 - DNA, 37 bp, Artificial Sequence
  Synthetic Oligonucleotide
tgcctcaggcttaggcataataggtatgtatcgaggg

SEQ ID NO: 175 - DNA, 37 bp, Artificial Sequence
  Synthetic Oligonucleotide
tgcctcaggcttaggcataatcggtatgtatcgcggg

SEQ ID NO: 176 - DNA, 37 bp, Artificial Sequence
  Synthetic Oligonucleotide
tgcctcaggcttaggcataataggtatgtatcgcggg

SEQ ID NO: 177 - DNA, 28 bp, Artificial Sequence
  Synthetic Oligonucleotide
ctgctgcwgaaaatagytctgtgtttgg

SEQ ID NO: 178 - DNA, 24 bp, Artificial Sequence
  Synthetic Oligonucleotide
tgctgaaaatagttctgtgtttgg